European Patent Specification EP 3 825 692 B1, published September 4, 2024. Title: METHOD FOR THE PROGNOSIS AND TREATMENT OF CANCER METASTASIS. Applicant: InBioMotion, S.L. Gomis, Roger Pavlovic, Milica Planet, Evarist Arnal, Anna Tarragona, Maria. The sequence listing filed with the application follows.

SEQUENCE LISTING (13 sequences)

SEQ ID NO: 1 - DNA, 6878 bp, Homo sapiens
agaggctttaaaatcttttttcatcttctagctgtagctcgggctgcttgtcggcttggcctccccctcccccctttgctctctgcctcgtctttccccaggacttcgctattttgcttttttaaaaaaaggcaagaaagaactaaactcccccctccctctcctccagtcgggctgcacctctgccttgcactttgcacagaggtagagagcgcgcgagggagagagaggaaagaaaaaaaataataaagagagccaagcagaagaggaggcgagaagcatgaagtgttaactcccccgtgccaaggcccgcgccgcccggacagacgcccgccgcgcctccagccccgagcggacgccgcgcgcgccctgcctgcagcccgggccggcgaggcgagcccttccttatgcaaagcgcgcagcggagcggcgagcgggggacgccgcgcaccgggccgggctcctccagcttcgccgccgcagccaccaccgccgccaccgcagctcgcggaggatcttcccgagcctgaagccgccggctcggcgcgcaaggaggcgagcgagcaaggaggggccggggcgagcgagggagcacattggcgtgagcaggggggagggagggcgggcgcggggggcgcgggcagggcgggggggtgtgtgtgtgagcgcgctcggaggtttcgggccagccaccgccgcgcaagctagaagcgccccagcccggcaagctggctcacccgctggccacccagcacagcccgctggcccctctcctgcagcccatctggcggagcggcggcggcggcggcggcggcggcaggagaatggcatcagaactggcaatgagcaactccgacctgcccaccagtcccctggccatggaatatgttaatgacttcgatctgatgaagtttgaagtgaaaaaggaaccggtggagaccgaccgcatcatcagccagtgcggccgtctcatcgccgggggctcgctgtcctccacccccatgagcacgccgtgcagctcggtgcccccttcccccagcttctcggcgcccagcccgggctcgggcagcgagcagaaggcgcacctggaagactactactggatgaccggctacccgcagcagctgaaccccgaggcgctgggcttcagccccgaggacgcggtcgaggcgctcatcagcaacagccaccagctccagggcggcttcgatggctacgcgcgcggggcgcagcagctggccgcggcggccggggccggtgccggcgcctccttgggcggcagcggcgaggagatgggccccgccgccgccgtggtgtccgccgtgatcgccgcggccgccgcgcagagcggcgcgggcccgcactaccaccaccaccaccaccacgccgccggccaccaccaccacccgacggccggcgcgcccggcgccgcgggcagcgcggccgcctcggccggtggcgctgggggcgcgggcggcggtggcccggccagcgctgggggcggcggcggcggcggcggcggcggaggcggcgggggcgcggcgggggcggggggcgccctgcacccgcaccacgccgccggcggcctgcacttcgacgaccgcttctccgacgagcagctggtgaccatgtctgtgcgcgagctgaaccggcagctgcgcggggtcagcaaggaggaggtgatccggctgaagcagaagaggcggaccctgaaaaaccgcggctatgcccagtcctgccgcttcaagagggtgcagcagagacacgtcctggagtcggagaagaaccagctgctgcagcaagtcgaccacctcaagcaggagatctccaggctggtgcgcgagagggacgcgtacaaggagaaatacgagaagttggtgagcagcggcttccgagaaaacggctcgagcagcgacaacccgtcctctcccgagtttttcatgtgagtctgacacgcgattccagctagccaccctgataagtgctccgcgggggtccggctcgggtgtgggcttgctagttctagagccatgctcgccaccacctcaccacccccacccccaccgagtttggcccccttggccccctacacacacacaaacccgcacgcacacaccacacacacacacacacacacacacacaccccacaccctgctcgagtttgtggtggtggtggctgttttaaactggggagggaatgggtgtctggctcatggattgccaatctgaaattctccataacttgctagcttgttttttttttttttttacacccccccgccccacccccggacttgcacaatgttcaatgatctcagcagagttcttcatgtgaaacgttgatcacctttgaagcctgcatcattcacatattttttcttcttcttccccttcagttcatgaactggtgttcattttctgtgtgtgtgtgtgttttattttgtttggatttttttttttaattttacttttagagcttgctgtgttgcccaccttttttccaacctccaccctcactccttctcaacccatctcttccgagatgaaagaaaaaaaaaagcaaagtttttttttcttctcctgagttcttcatgtgagattgagcttgcaaaggaaaaaaaaatgtgaaatgttatagacttgcagcgtgccgagttccatcgggttttttttttagcattgttatgctaaaatagagaaaaaaatcctcatgaaccttccacaatcaagcctgcatcaaccttctgggtgtgacttgtgagttttggccttgtgatgccaaatctgagagtttagtctgccattaaaaaaactcattctcatctcatgcattattatgcttgctactttgtcttagcaacaatgaactataactgtttcaaagactttatggaaaagagacattatattaataaaaaaaaaaagcctgcatgctggacatgtatggtataattattttttcctttttttttccttttggcttggaaatggacgttcgaagacttatagcatggcattcatacttttgttttattgcctcatgacttttttgagtttagaacaaaacagtgcaaccgtagagccttcttcccatgaaattttgcatctgctccaaaactgctttgagttactcagaacttcaacctcccaatgcactgaaggcattccttgtcaaagataccagaatgggttacacatttaacctggcaaacattgaagaactcttaatgttttctttttaataagaatgacgccccactttggggactaaaattgtgctattgccgagaagcagtctaaaatttattttttaaaaagagaaactgccccattatttttggtttgttttatttttattttatattttttggcttttggtcattgtcaaatgtggaatgctctgggtttctagtatataatttaattctagtttttataatctgttagcccagttaaaatgtatgctacagataaaggaatgttatagataaatttgaaagagttaggtctgtttagctgtagattttttaaacgattgatgcactaaattgtttactattgtgatgttaaggggggtagagtttgcaaggggactgtttaaaaaaagtagcttatacagcatgtgcttgcaacttaaatataagttgggtatgtgtagtctttgctataccactgactgtattgaaaaccaaagtattaagaggggaaacgcccctgtttatatctgtaggggtattttacattcaaaaatgtatgtttttttttcttttcaaaattaaagtatttgggactgaattgcactaagatataacctgcaagcatataatacaaaaaaaaattgcaaaactgtttagaacgctaataaaatttatgcagttataaaaatggcattactgcacagttttaagatgatgcagatttttttacagttgtattgtggtgcagaactggattttctgtaacttaaaaaaaaatccacagttttaaaggcaataatcagtaaatgttattttcagggactgacatcctgtctttaaaaagaaatgaaaagtaaatcttaccacaataaatataaaaaaatcttgtcagttacttttcttttacatattttgctgtgcaaaattgttttatatcttgagttactaactaaccacgcgtgttgttcctatgtgcttttctttcattttcaattctggttatatcaagaaaagaataatctacaataataaacggcatttttttttgattctgtactcagtttcttagtgtacagtttaactgggcccaacaacctcgttaaaagtgtaaaatgcatccttttctccagtggaaggattcctggaggaatagggagacagtaattcagggtgaaattataggctgttttttgaagtgaggaggctggccccatatactgattagcaatatttaatatagatgtaaattatgacctcatttttttctccccaaagttttcagttttcaaatgagttgagccataattgcccttggtaggaaaaacaaaacaaaacagtggaactaggcttcctgagcatggccctacacttctgatcaggagcaaagccatccatagacagaggagccggacaaatatggcgcatcagaggtggcttgcgcacatatgcattgaacggtaaagagaaacagcgcttgccttttcactaaagttgactatttttccttcttctcttacacaccgagattttcttgttagcaaggcctgacaagatttaacataaacatgacaaatcatagttgtttgttttgttttgcttttctctttaacactgaagatcatttgtcttaaataggaaaaagaaaatccactccttacttccatatttccaagtacatatctggtttaaactatgttatcaaatcatatttcaccgtgaatattcagtggagaacttctctacctggatgagctagtaatgatttcagatcatgctatccccagaaataaaagcaaaaaataatacctgtgtggaatataggctgtgctttgatttactggtatttaccccaaaataggctgtgtatgggggctgacttaaagatcccttggaaagactcaaaactaccttcactagtaggactcctaagcgctgacctatttttaaatgacacaaattcatgaaactaatgttacaaattcatgcagtttgcactcttagtcatcttcccctagcacaccaatagaatgttagacaaagccagcactgttttgaaaatacagccaaacacgatgacttttgttttgttttctgccgttcttaaaagaaaaaaagataatattgcaactctgactgaaagacttatttttaagaaaacaggttgtgtttggtgctgctaagttctggccagtttatcatctggccttcctgcctattttttacaaaacacgaagacagtgtgtaacctcgacattttgaccttcctttatgtgctagtttagacaggctcctgaatccacacttaattttgcttaacaaaagtcttaatagtaaacctcccctcatgagcttgaagtcaagtgttcttgacttcagatatttctttcctttttttttttttttcctcatcacaactaagagatacacaaactctgaagaagcagaaatggagagaatgcttttaacaaaaaagcatctgatgaaagattttaggcaaacattctcaaaataagagtgatattctggatgtagttattgcagttatctcatgacaaatgaggcctggattggaaggaaaatatagttgtgtagaattaagcattttgataggaatctacaaggtagttgaatataataagcaggtttgggcccccaaactttagaaaatcaaatgcaaaggtgctggcaaaaatgaggtttgagtggctggctgtaagagaaggttaactcctagtaaaaggcatttttagaaataacaattactgaaaactttgaagtatagtgggagtagcaaacaaatacatgttttttttttcttacaaagaactcctaaatcctgagtaagtgccattcattacaataagtctctaaatttaaaaaaaaaaaaatcatatgaggaaatctagctttcccctttacgctgcgtttgatctttgtctaaatagtgttaaaattcctttcattccaattacagaactgagcccactcgcaagttggagccatcagtgggatacgccacattttggaagccccagcatcgtgtacttaccagtgtgttcacaaaatgaaatttgtgtgagagctgtacattaaaaaaaatcatcattattattattatttgcagtcatggagaaccacctacccctgacttctgtttagtctcctttttaaataaaaattactgtgttagagaagaaggctattaaatgtagtagttaactatgcctcttgtctgggggtttcatagagaccggtaggaaagcgcactcctgcttttcgatttatggtgtgtgcaagtaaacaggtgcattgctttcaacctgccatactagttttaaaaattcactgaaattacaaagatacatatatatgcatatatataatggaaagtttcccggaatgcaacaattagcattttaaaatcatatataggcatgcacattctaaatagtactttttcatgcttcattgtttctctggcagataattttactaagaagaaaaatagatattcgactccccttccctaaacaaatccacgggcagaggctccagcggagccgagccccctggttttctcgtaggccctagacggtgttgcatttatcagtgatgtcaaacgtgctcatttgtcagacatagctgtaaatgaaaacaatgtgtggcaaaatacaaagtt

SEQ ID NO: 2 - DNA, 2656 bp, Homo sapiens
gaggctttaaaatcttttttcatcttctagctgtagctcgggctgcttgtcggcttggcctccccctcccccctttgctctctgcctcgtctttccccaggacttcgctattttgcttttttaaaaaaaggcaagaaagaactaaactcccccctccctctcctccagtcgggctgcacctctgccttgcactttgcacagaggtagagagcgcgcgagggagagagaggaaagaaaaaaaataataaagagagccaagcagaagaggaggcgagaagcatgaagtgttaactcccccgtgccaaggcccgcgccgcccggacagacgcccgccgcgcctccagccccgagcggacgccgcgcgcgccctgcctgcagcccgggccggcgaggcgagcccttccttatgcaaagcgcgcagcggagcggcgagcgggggacgccgcgcaccgggccgggctcctccagcttcgccgccgcagccaccaccgccgccaccgcagctcgcggaggatcttcccgagcctgaagccgccggctcggcgcgcaaggaggcgagcgagcaaggaggggccggggcgagcgagggagcacattggcgtgagcaggggggagggagggcgggcgcggggggcgcgggcagggcgggggggtgtgtgtgtgagcgcgctcggaggtttcgggccagccaccgccgcgcaagctagaagcgccccagcccggcaagctggctcacccgctggccacccagcacagcccgctggcccctctcctgcagcccatctggcggagcggcggcggcggcggcggcggcggcaggagaatggcatcagaactggcaatgagcaactccgacctgcccaccagtcccctggccatggaatatgttaatgacttcgatctgatgaagtttgaagtgaaaaaggaaccggtggagaccgaccgcatcatcagccagtgcggccgtctcatcgccgggggctcgctgtcctccacccccatgagcacgccgtgcagctcggtgcccccttcccccagcttctcggcgcccagcccgggctcgggcagcgagcagaaggcgcacctggaagactactactggatgaccggctacccgcagcagctgaaccccgaggcgctgggcttcagccccgaggacgcggtcgaggcgctcatcagcaacagccaccagctccagggcggcttcgatggctacgcgcgcggggcgcagcagctggccgcggcggccggggccggtgccggcgcctccttgggcggcagcggcgaggagatgggccccgccgccgccgtggtgtccgccgtgatcgccgcggccgccgcgcagagcggcgcgggcccgcactaccaccaccaccaccaccacgccgccggccaccaccaccacccgacggccggcgcgcccggcgccgcgggcagcgcggccgcctcggccggtggcgctgggggcgcgggcggcggtggcccggccagcgctgggggcggcggcggcggcggcggcggcggaggcggcgggggcgcggcgggggcggggggcgccctgcacccgcaccacgccgccggcggcctgcacttcgacgaccgcttctccgacgagcagctggtgaccatgtctgtgcgcgagctgaaccggcagctgcgcggggtcagcaaggaggaggtgatccggctgaagcagaagaggcggaccctgaaaaaccgcggctatgcccagtcctgccgcttcaagagggtgcagcagagacacgtcctggagtcggagaagaaccagctgctgcagcaagtcgaccacctcaagcaggagatctccaggctggtgcgcgagagggacgcgtacaaggagaaatacgagaagttggtgagcagcggcttccgagaaaacggctcgagcagcgacaacccgtcctctcccgagtttttcataactgagcccactcgcaagttggagccatcagtgggatacgccacattttggaagccccagcatcgtgtacttaccagtgtgttcacaaaatgaaatttgtgtgagagctgtacattaaaaaaaatcatcattattattattatttgcagtcatggagaaccacctacccctgacttctgtttagtctcctttttaaataaaaattactgtgttagagaagaaggctattaaatgtagtagttaactatgcctcttgtctgggggtttcatagagaccggtaggaaagcgcactcctgcttttcgatttatggtgtgtgcaagtaaacaggtgcattgctttcaacctgccatactagttttaaaaattcactgaaattacaaagatacatatatatgcatatatataatggaaagtttcccggaatgcaacaattagcattttaaaatcatatataggcatgcacattctaaatagtactttttcatgcttcattgtttctctggcagataattttactaagaagaaaaatagatattcgactccccttccctaaacaaatccacgggcagaggctccagcggagccgagccccctggttttctcgtaggccctagacggtgttgcatttatcagtgatgtcaaacgtgctcatttgtcagacatagctgtaaatgaaaacaatgtgtggcaaaatacaaagttaaaaaaaaaa

SEQ ID NO: 3 - DNA, 6887 bp, Homo sapiens
gaggctttaaaatcttttttcatcttctagctgtagctcgggctgcttgtcggcttggcctccccctcccccctttgctctctgcctcgtctttccccaggacttcgctattttgcttttttaaaaaaaggcaagaaagaactaaactcccccctccctctcctccagtcgggctgcacctctgccttgcactttgcacagaggtagagagcgcgcgagggagagagaggaaagaaaaaaaataataaagagagccaagcagaagaggaggcgagaagcatgaagtgttaactcccccgtgccaaggcccgcgccgcccggacagacgcccgccgcgcctccagccccgagcggacgccgcgcgcgccctgcctgcagcccgggccggcgaggcgagcccttccttatgcaaagcgcgcagcggagcggcgagcgggggacgccgcgcaccgggccgggctcctccagcttcgccgccgcagccaccaccgccgccaccgcagctcgcggaggatcttcccgagcctgaagccgccggctcggcgcgcaaggaggcgagcgagcaaggaggggccggggcgagcgagggagcacattggcgtgagcaggggggagggagggcgggcgcggggggcgcgggcagggcgggggggtgtgtgtgtgagcgcgctcggaggtttcgggccagccaccgccgcgcaagctagaagcgccccagcccggcaagctggctcacccgctggccacccagcacagcccgctggcccctctcctgcagcccatctggcggagcggcggcggcggcggcggcggcggcaggagaatggcatcagaactggcaatgagcaactccgacctgcccaccagtcccctggccatggaatatgttaatgacttcgatctgatgaagtttgaagtgaaaaaggaaccggtggagaccgaccgcatcatcagccagtgcggccgtctcatcgccgggggctcgctgtcctccacccccatgagcacgccgtgcagctcggtgcccccttcccccagcttctcggcgcccagcccgggctcgggcagcgagcagaaggcgcacctggaagactactactggatgaccggctacccgcagcagctgaaccccgaggcgctgggcttcagccccgaggacgcggtcgaggcgctcatcagcaacagccaccagctccagggcggcttcgatggctacgcgcgcggggcgcagcagctggccgcggcggccggggccggtgccggcgcctccttgggcggcagcggcgaggagatgggccccgccgccgccgtggtgtccgccgtgatcgccgcggccgccgcgcagagcggcgcgggcccgcactaccaccaccaccaccaccacgccgccggccaccaccaccacccgacggccggcgcgcccggcgccgcgggcagcgcggccgcctcggccggtggcgctgggggcgcgggcggcggtggcccggccagcgctgggggcggcggcggcggcggcggcggcggaggcggcgggggcgcggcgggggcggggggcgccctgcacccgcaccacgccgccggcggcctgcacttcgacgaccgcttctccgacgagcagctggtgaccatgtctgtgcgcgagctgaaccggcagctgcgcggggtcagcaaggaggaggtgatccggctgaagcagaagaggcggaccctgaaaaaccgcggctatgcccagtcctgccgcttcaagagggtgcagcagagacacgtcctggagtcggagaagaaccagctgctgcagcaagtcgaccacctcaagcaggagatctccaggctggtgcgcgagagggacgcgtacaaggagaaatacgagaagttggtgagcagcggcttccgagaaaacggctcgagcagcgacaacccgtcctctcccgagtttttcatgtgagtctgacacgcgattccagctagccaccctgataagtgctccgcgggggtccggctcgggtgtgggcttgctagttctagagccatgctcgccaccacctcaccacccccacccccaccgagtttggcccccttggccccctacacacacacaaacccgcacgcacacaccacacacacacacacacacacacacacaccccacaccctgctcgagtttgtggtggtggtggctgttttaaactggggagggaatgggtgtctggctcatggattgccaatctgaaattctccataacttgctagcttgttttttttttttttttacacccccccgccccacccccggacttgcacaatgttcaatgatctcagcagagttcttcatgtgaaacgttgatcacctttgaagcctgcatcattcacatattttttcttcttcttccccttcagttcatgaactggtgttcattttctgtgtgtgtgtgtgttttattttgtttggatttttttttttaattttacttttagagcttgctgtgttgcccaccttttttccaacctccaccctcactccttctcaacccatctcttccgagatgaaagaaaaaaaaaagcaaagtttttttttcttctcctgagttcttcatgtgagattgagcttgcaaaggaaaaaaaaatgtgaaatgttatagacttgcagcgtgccgagttccatcgggttttttttttagcattgttatgctaaaatagagaaaaaaatcctcatgaaccttccacaatcaagcctgcatcaaccttctgggtgtgacttgtgagttttggccttgtgatgccaaatctgagagtttagtctgccattaaaaaaactcattctcatctcatgcattattatgcttgctactttgtcttagcaacaatgaactataactgtttcaaagactttatggaaaagagacattatattaataaaaaaaaaaagcctgcatgctggacatgtatggtataattattttttcctttttttttccttttggcttggaaatggacgttcgaagacttatagcatggcattcatacttttgttttattgcctcatgacttttttgagtttagaacaaaacagtgcaaccgtagagccttcttcccatgaaattttgcatctgctccaaaactgctttgagttactcagaacttcaacctcccaatgcactgaaggcattccttgtcaaagataccagaatgggttacacatttaacctggcaaacattgaagaactcttaatgttttctttttaataagaatgacgccccactttggggactaaaattgtgctattgccgagaagcagtctaaaatttattttttaaaaagagaaactgccccattatttttggtttgttttatttttattttatattttttggcttttggtcattgtcaaatgtggaatgctctgggtttctagtatataatttaattctagtttttataatctgttagcccagttaaaatgtatgctacagataaaggaatgttatagataaatttgaaagagttaggtctgtttagctgtagattttttaaacgattgatgcactaaattgtttactattgtgatgttaaggggggtagagtttgcaaggggactgtttaaaaaaagtagcttatacagcatgtgcttgcaacttaaatataagttgggtatgtgtagtctttgctataccactgactgtattgaaaaccaaagtattaagaggggaaacgcccctgtttatatctgtaggggtattttacattcaaaaatgtatgtttttttttcttttcaaaattaaagtatttgggactgaattgcactaagatataacctgcaagcatataatacaaaaaaaaattgcaaaactgtttagaacgctaataaaatttatgcagttataaaaatggcattactgcacagttttaagatgatgcagatttttttacagttgtattgtggtgcagaactggattttctgtaacttaaaaaaaaatccacagttttaaaggcaataatcagtaaatgttattttcagggactgacatcctgtctttaaaaagaaatgaaaagtaaatcttaccacaataaatataaaaaaatcttgtcagttacttttcttttacatattttgctgtgcaaaattgttttatatcttgagttactaactaaccacgcgtgttgttcctatgtgcttttctttcattttcaattctggttatatcaagaaaagaataatctacaataataaacggcatttttttttgattctgtactcagtttcttagtgtacagtttaactgggcccaacaacctcgttaaaagtgtaaaatgcatccttttctccagtggaaggattcctggaggaatagggagacagtaattcagggtgaaattataggctgttttttgaagtgaggaggctggccccatatactgattagcaatatttaatatagatgtaaattatgacctcatttttttctccccaaagttttcagttttcaaatgagttgagccataattgcccttggtaggaaaaacaaaacaaaacagtggaactaggcttcctgagcatggccctacacttctgatcaggagcaaagccatccatagacagaggagccggacaaatatggcgcatcagaggtggcttgcgcacatatgcattgaacggtaaagagaaacagcgcttgccttttcactaaagttgactatttttccttcttctcttacacaccgagattttcttgttagcaaggcctgacaagatttaacataaacatgacaaatcatagttgtttgttttgttttgcttttctctttaacactgaagatcatttgtcttaaataggaaaaagaaaatccactccttacttccatatttccaagtacatatctggtttaaactatgttatcaaatcatatttcaccgtgaatattcagtggagaacttctctacctggatgagctagtaatgatttcagatcatgctatccccagaaataaaagcaaaaaataatacctgtgtggaatataggctgtgctttgatttactggtatttaccccaaaataggctgtgtatgggggctgacttaaagatcccttggaaagactcaaaactaccttcactagtaggactcctaagcgctgacctatttttaaatgacacaaattcatgaaactaatgttacaaattcatgcagtttgcactcttagtcatcttcccctagcacaccaatagaatgttagacaaagccagcactgttttgaaaatacagccaaacacgatgacttttgttttgttttctgccgttcttaaaagaaaaaaagataatattgcaactctgactgaaagacttatttttaagaaaacaggttgtgtttggtgctgctaagttctggccagtttatcatctggccttcctgcctattttttacaaaacacgaagacagtgtgtaacctcgacattttgaccttcctttatgtgctagtttagacaggctcctgaatccacacttaattttgcttaacaaaagtcttaatagtaaacctcccctcatgagcttgaagtcaagtgttcttgacttcagatatttctttcctttttttttttttttcctcatcacaactaagagatacacaaactctgaagaagcagaaatggagagaatgcttttaacaaaaaagcatctgatgaaagattttaggcaaacattctcaaaataagagtgatattctggatgtagttattgcagttatctcatgacaaatgaggcctggattggaaggaaaatatagttgtgtagaattaagcattttgataggaatctacaaggtagttgaatataataagcaggtttgggcccccaaactttagaaaatcaaatgcaaaggtgctggcaaaaatgaggtttgagtggctggctgtaagagaaggttaactcctagtaaaaggcatttttagaaataacaattactgaaaactttgaagtatagtgggagtagcaaacaaatacatgttttttttttcttacaaagaactcctaaatcctgagtaagtgccattcattacaataagtctctaaatttaaaaaaaaaaaaatcatatgaggaaatctagctttcccctttacgctgcgtttgatctttgtctaaatagtgttaaaattcctttcattccaattacagaactgagcccactcgcaagttggagccatcagtgggatacgccacattttggaagccccagcatcgtgtacttaccagtgtgttcacaaaatgaaatttgtgtgagagctgtacattaaaaaaaatcatcattattattattatttgcagtcatggagaaccacctacccctgacttctgtttagtctcctttttaaataaaaattactgtgttagagaagaaggctattaaatgtagtagttaactatgcctcttgtctgggggtttcatagagaccggtaggaaagcgcactcctgcttttcgatttatggtgtgtgcaagtaaacaggtgcattgctttcaacctgccatactagttttaaaaattcactgaaattacaaagatacatatatatgcatatatataatggaaagtttcccggaatgcaacaattagcattttaaaatcatatataggcatgcacattctaaatagtactttttcatgcttcattgtttctctggcagataattttactaagaagaaaaatagatattcgactccccttccctaaacaaatccacgggcagaggctccagcggagccgagccccctggttttctcgtaggccctagacggtgttgcatttatcagtgatgtcaaacgtgctcatttgtcagacatagctgtaaatgaaaacaatgtgtggcaaaatacaaagttaaaaaaaaaa

SEQ ID NO: 4 - protein, 403 aa, Homo sapiens
MASELAMSNSDLPTSPLAMEYVNDFDLMKFEVKKEPVETDRIISQCGRLIAGGSLSSTPMSTPCSSVPPSPSFSAPSPGSGSEQKAHLEDYYWMTGYPQQLNPEALGFSPEDAVEALISNSHQLQGGFDGYARGAQQLAAAAGAGAGASLGGSGEEMGPAAAVVSAVIAAAAAQSGAGPHYHHHHHHAAGHHHHPTAGAPGAAGSAAASAGGAGGAGGGGPASAGGGGGGGGGGGGGGAAGAGGALHPHHAAGGLHFDDRFSDEQLVTMSVRELNRQLRGVSKEEVIRLKQKRRTLKNRGYAQSCRFKRVQQRHVLESEKNQLLQQVDHLKQEISRLVRERDAYKEKYEKLVSSGFRENGSSSDNPSSPEFFITEPTRKLEPSVGYATFWKPQHRVLTSVFTK

SEQ ID NO: 5 - protein, 373 aa, Homo sapiens
MASELAMSNSDLPTSPLAMEYVNDFDLMKFEVKKEPVETDRIISQCGRLIAGGSLSSTPMSTPCSSVPPSPSFSAPSPGSGSEQKAHLEDYYWMTGYPQQLNPEALGFSPEDAVEALISNSHQLQGGFDGYARGAQQLAAAAGAGAGASLGGSGEEMGPAAAVVSAVIAAAAAQSGAGPHYHHHHHHAAGHHHHPTAGAPGAAGSAAASAGGAGGAGGGGPASAGGGGGGGGGGGGGGAAGAGGALHPHHAAGGLHFDDRFSDEQLVTMSVRELNRQLRGVSKEEVIRLKQKRRTLKNRGYAQSCRFKRVQQRHVLESEKNQLLQQVDHLKQEISRLVRERDAYKEKYEKLVSSGFRENGSSSDNPSSPEFFM

SEQ ID NO: 6 - RNA, 19 nt, Artificial Sequence
  c-MAF specific siRNA
acggcucgagcagcgacaa

SEQ ID NO: 7 - RNA, 19 nt, Artificial Sequence
  c-MAF specific siRNA
cuuaccaguguguucacaa

SEQ ID NO: 8 - RNA, 20 nt, Artificial Sequence
  c-MAF specific siRNA
uggaagacuacuacuggaug

SEQ ID NO: 9 - RNA, 20 nt, Artificial Sequence
  c-MAF specific siRNA
auuugcagucauggagaacc

SEQ ID NO: 10 - RNA, 20 nt, Artificial Sequence
  c-MAF specific siRNA
caaggagaaauacgagaagu

SEQ ID NO: 11 - RNA, 20 nt, Artificial Sequence
  c-MAF specific siRNA
acaaggagaaauacgagaag

SEQ ID NO: 12 - RNA, 20 nt, Artificial Sequence
  c-MAF specific siRNA
accuggaagacuacuacugg

SEQ ID NO: 13 - DNA, 13878 bp, Homo sapiens
aactatatattaaacacctccggtctgagaggccgtgttgggtgtctttgtcaggtgaagaaagagaagaaggctggtacaccttcccaggaattctcactgaagaaaacatctggattttttacatctcttgtgcaaaacaaacaaagatttcattaagtgatgtatattgttttccaaggaagaaacctgcagagacaaaaacaaataagcaaataattgaaacaaaaatatgataaacccccaaattcttccagtgctaatttacttgttatcatggttctctacaaaggcagagatcactaattacaggtttttccagaattcacatttcacgtcaagatcatccaatccaaacagtgtacggaaagcctagggccttcttcactttgccccctaccccaccctacacacacgcccccatctaaatgatacccttggaaagaaacctacacatctcatttgtctatattttgcttcctccctcgcctcccggtaaccaaatgtgagttgttctctaactgcactggagaatcagaatttattgtacatatgtttgtgttccacttaataaaaaaacctatattttaagataaactttgttagtaattcatgaggtaagtgactatttatgctaatcaggcagaaatatattctcaagcataatgcattacataaatttgaatgtaaaatgttcaattatgaagtaaatacaggtaatgcaaataataaattacctctaataaaaattataaaagatgtgccttgaaagagagagcggctttaacttacaactgtgaattgcttaaagagaaaagaattaataaatgctgaattactctgatgattatttagcacataattcacctattcataacgactcctagtaatcagactgttgtttcacatcctccaacatgaggcaagactgtttcctcagcaattttgcccttatcagattatctcgtctgattctattaattttcttccatgaatctgctaacagtgatttgtgatttacttaccctgctaactgaagactgttaaaaggatttatctaacactggacctaagaacagtgtacgccttatcgttcagttactctgaagaactctttctcaaatcaatttagttggtttcatagtgaaatttagtggacactggttagttctgccccataaaatcagcccctaaacaaagagtccagacaccatacctgatgcatcccattctattcagattatggatgtctgattccaacatgatatatttgagttgctataactcacaatcggggaaaatatattcctttaagcttttaatctttgtaatttggacatgaacaggggttttgtttttcatttttgcatgaagtcattatgtatgtactgacgtgaaactataattgtgtttctgatgttactgtgtcacaatattctatgcgatgtaacccatgtcctcctccccctcacaaatctcctataaatattcattgctttcaaaaactttaatactactggtccgaattggtcaataatgacaaatgcatggtttctaaattactgtatattgttctacagagattactagagtatatatagcaaggggatgttaagcagtaagaaaacacagttcacattgtatttggattagattggcttggatagaagtgaaacaaacaatgttagcaaagaagtctaaagacatgtggcccactgtaattgtacagaatcaaaaacctgaatagtactcattaaaatgagagagctcaattgttataaaagaaatgctgctaacagagaactgtaaatgtttagacacccctgtgaatcactaaataataatgtaaaaaggataaaaatgagaattaagttataagcctgagagcattactgctacacatctaaaaaaataattctgatcctctcttttttttttccaagagaaaatgggcgactataaaagaccttgcaataagagaaataaaaataccatgtcttcacagcagtgtacataaataaaccataaaaatgtgcagataataatatatttagctgcccaaacatgggcatttaatttctagaaatgatatataacaatgtaacaattagatactcagccatgaatgtgtatggcacagtcttcatcattagcaaactttgtgtataaaatattatttattatttattataatactgctttcagaggcaatgatcataccttacagcttttaacacaaatatgatgcaaaaggattaaaagtatatcataaacaaacaataaattctttctaaatacacttaaattcatattttacatgaaaaatataaacttcctacatttgtgactactgacttttaaaaagacctagaaaactattgttacgggcaatgttaaatgacataatgcttatgtaatggaaagtgtggattttcctctaaataaactataatcccttaacttcattactagggaaaatattgttaaagagaaggaaagcaagggaattctgctaggttgcataaatattgacataatcttcactctttcttccccaaactggtaatagacatagtttattccacccaacaaaatgctcttataagaccaaaactacccttattaacaacttctctgcagtcacgatgaaaagaaacactacttgtctgaaaaataccgacagcgctgcccttttcagattagggtgtgcctacgaatcttttgggaagtcttccattaaggattcctgggtttgctgaaactgaagtctactaggatcagagaaattaacacaggtctaatatggtgcaaggaacgagtgagagacacctgaggttataaatagcaaagcatgctgcggggtggggaagaccattctgaagtgcaatgttcaagacgctggcttaatatatgactaagtgtcagaagtcaggttttctgagaattactttccagataaacaactttatagcactgcacttaatcttacttactagagacatctcatttatcactgaattacaagtaactttaatcctattgatattgccataaagcccgttgaaaatccatcctggcacttttaaagggtttggggccctgttacatggggatcctcttgcaaaggtctcagccagaaattacaccccgagggtgtctgtatcccctggcctctttgtcaacaatcaaggagaagaggaggggcaaaaatgatctctgcatctgccagcactttcttcggcccctttcctatagggtcgggttctcccacttcagtcaaactaactttgtgtgtctctttcctcctcccacactgggtaaccagctgcttttcacttcatcgacaaaactggacacggatcaatttcaactgacctttgccgaaaggtggcgctgttgaggtaaaaaccaactcgctccaacaatagtttccactcttcgatccttttgcaggcttttcagaatttttttttttttttaatgcaccctcctagcgtctcccccttctcataaagtaaaataaatacgattaaaaacaccaaatgcatttcattaattgaaggaatcaacagtcccaacttctaagcagacgggctggtcttccaaaggctgggtcggtttcaggagctttctctccaaataaatctctgcttcttcgacttgcctatcgctttaaaatcttagaaacagagttagttgttggtttccttcttttttctttttcttttttatttcttttttgcataaacttttagagaatcaatctagaaatttgaactacttattagcatttgcaactgggggtggggggagcagcctcccccaccccaccccccactctgcgtttccggactagttccagaaaccgcggtttaaaatttaacccttcgagggtagctggtgagggctggggtattgtttttcccccttgctccctgccacgatcaagtccgaaataattaaaggaaacgtaaaagtgcaaagggcgcgcctgaccctgataaacagaggtcagatttcgtaaggggacgggtgagtgtgagtgtgtgtgtgtttgtgtgtgtgtgtgtaagagagagagagagcgagcgcgcaatatgagtctcaaaggccaaactccggccagtcaggagccggaaggctgagcccggctgacctgactttgagcttccccggagttatctcgcataggcgctcgctctgtccaagggcacgcgacgccagcgggcagccggtctccgtgaagaatggcctctaaacaacttattttacctcgttgtaaagagagggataaaatgggctttccctctccacggatgcccagccttctgggcaggcgcatggccgggcggcgcccagcccgcagccccgatccggacaccccactgcatccctcccttcccggtcccttccccgcacgggcgcccgagagacggacaaagagttggggccaagtttgagcgccgggcacggccaggctcagggaaggaaggtccccggcagacacctgggtaccagagttggtgcgaggaggaaaagctgggaggcgaattcacaatcctgggggtggagggcaggcaggggaggggaatcaggccaatcccagccgagtgagcccccagcgagctggggctccggatgggaggcctgtctcgcgctccaaagaaaagcaaaccgccctcccaggtccgcccggattgccgaagcccctctggaaaaactccttcccctcttacaccaaactttgcgccgggcctcgttccctcccgggtaggcagcggcgcaggaagggttaagccagcccgtcccagctgacagtcagctgattgggccctgattgacagctccgaaaagtttccttgtttctatactattatgctaatcgcggccgctctcgccgcctcccattggcccggagtgccagtcaatttctcatttggacctgacgtcacgagtgctataaaactcagcaattgctttaaactcttcttgctggatcagaggctttaaaatcttttttcatcttctagctgtagctcgggctgcttgtcggcttggcctccccctcccccctttgctctctgcctcgtctttccccaggacttcgctattttgcttttttaaaaaaaggcaagaaagaactaaactcccccctccctctcctccagtcgggctgcacctctgccttgcactttgcacagaggtagagagcgcgcgagggagagagaggaaagaaaaaaaataataaagagagccaagcagaagaggaggcgagaagcatgaagtgttaactcccccgtgccaaggcccgcgccgcccggacagacgcccgccgcgcctccagccccgagcggacgccgcgcgcgccctgcctgcagcccgggccggcgaggcgagcccttccttatgcaaagcgcgcagcggagcggcgagcgggggacgccgcgcaccgggccgggctcctccagcttcgccgccgcagccaccaccgccgccaccgcagctcgcggaggatcttcccgagcctgaagccgccggctcggcgcgcaaggaggcgagcgagcaaggaggggccggggcgagcgagggagcacattggcgtgagcaggggggagggagggcgggcgcggggggcgcgggcagggcgggggggtgtgtgtgtgagcgcgctcggaggtttcgggccagccaccgccgcgcaagctagaagcgccccagcccggcaagctggctcacccgctggccacccagcacagcccgctggcccctctcctgcagcccatctggcggagcggcggcggcggcggcggcggcggcaggagaatggcatcagaactggcaatgagcaactccgacctgcccaccagtcccctggccatggaatatgttaatgacttcgatctgatgaagtttgaagtgaaaaaggaaccggtggagaccgaccgcatcatcagccagtgcggccgtctcatcgccgggggctcgctgtcctccacccccatgagcacgccgtgcagctcggtgcccccttcccccagcttctcggcgcccagcccgggctcgggcagcgagcagaaggcgcacctggaagactactactggatgaccggctacccgcagcagctgaaccccgaggcgctgggcttcagccccgaggacgcggtcgaggcgctcatcagcaacagccaccagctccagggcggcttcgatggctacgcgcgcggggcgcagcagctggccgcggcggccggggccggtgccggcgcctccttgggcggcagcggcgaggagatgggccccgccgccgccgtggtgtccgccgtgatcgccgcggccgccgcgcagagcggcgcgggcccgcactaccaccaccaccaccaccacgccgccggccaccaccaccacccgacggccggcgcgcccggcgccgcgggcagcgcggccgcctcggccggtggcgctgggggcgcgggcggcggtggcccggccagcgctgggggcggcggcggcggcggcggcggcggaggcggcgggggcgcggcgggggcggggggcgccctgcacccgcaccacgccgccggcggcctgcacttcgacgaccgcttctccgacgagcagctggtgaccatgtctgtgcgcgagctgaaccggcagctgcgcggggtcagcaaggaggaggtgatccggctgaagcagaagaggcggaccctgaaaaaccgcggctatgcccagtcctgccgcttcaagagggtgcagcagagacacgtcctggagtcggagaagaaccagctgctgcagcaagtcgaccacctcaagcaggagatctccaggctggtgcgcgagagggacgcgtacaaggagaaatacgagaagttggtgagcagcggcttccgagaaaacggctcgagcagcgacaacccgtcctctcccgagtttttcatgtgagtctgacacgcgattccagctagccaccctgataagtgctccgcgggggtccggctcgggtgtgggcttgctagttctagagccatgctcgccaccacctcaccacccccacccccaccgagtttggcccccttggccccctacacacacacaaacccgcacgcacacaccacacacacacacacacacacacacacaccccacaccctgctcgagtttgtggtggtggtggctgttttaaactggggagggaatgggtgtctggctcatggattgccaatctgaaattctccataacttgctagcttgttttttttttttttttacacccccccgccccacccccggacttgcacaatgttcaatgatctcagcagagttcttcatgtgaaacgttgatcacctttgaagcctgcatcattcacatattttttcttcttcttccccttcagttcatgaactggtgttcattttctgtgtgtgtgtgtgttttattttgtttggatttttttttttaattttacttttagagcttgctgtgttgcccaccttttttccaacctccaccctcactccttctcaacccatctcttccgagatgaaagaaaaaaaaaagcaaagtttttttttcttctcctgagttcttcatgtgagattgagcttgcaaaggaaaaaaaaatgtgaaatgttatagacttgcagcgtgccgagttccatcgggttttttttttagcattgttatgctaaaatagagaaaaaaatcctcatgaaccttccacaatcaagcctgcatcaaccttctgggtgtgacttgtgagttttggccttgtgatgccaaatctgagagtttagtctgccattaaaaaaactcattctcatctcatgcattattatgcttgctactttgtcttagcaacaatgaactataactgtttcaaagactttatggaaaagagacattatattaataaaaaaaaaaagcctgcatgctggacatgtatggtataattattttttcctttttttttccttttggcttggaaatggacgttcgaagacttatagcatggcattcatacttttgttttattgcctcatgacttttttgagtttagaacaaaacagtgcaaccgtagagccttcttcccatgaaattttgcatctgctccaaaactgctttgagttactcagaacttcaacctcccaatgcactgaaggcattccttgtcaaagataccagaatgggttacacatttaacctggcaaacattgaagaactcttaatgttttctttttaataagaatgacgccccactttggggactaaaattgtgctattgccgagaagcagtctaaaatttattttttaaaaagagaaactgccccattatttttggtttgttttatttttattttatattttttggcttttggtcattgtcaaatgtggaatgctctgggtttctagtatataatttaattctagtttttataatctgttagcccagttaaaatgtatgctacagataaaggaatgttatagataaatttgaaagagttaggtctgtttagctgtagattttttaaacgattgatgcactaaattgtttactattgtgatgttaaggggggtagagtttgcaaggggactgtttaaaaaaagtagcttatacagcatgtgcttgcaacttaaatataagttgggtatgtgtagtctttgctataccactgactgtattgaaaaccaaagtattaagaggggaaacgcccctgtttatatctgtaggggtattttacattcaaaaatgtatgtttttttttcttttcaaaattaaagtatttgggactgaattgcactaagatataacctgcaagcatataatacaaaaaaaaattgcaaaactgtttagaacgctaataaaatttatgcagttataaaaatggcattactgcacagttttaagatgatgcagatttttttacagttgtattgtggtgcagaactggattttctgtaacttaaaaaaaaatccacagttttaaaggcaataatcagtaaatgttattttcagggactgacatcctgtctttaaaaagaaatgaaaagtaaatcttaccacaataaatataaaaaaatcttgtcagttacttttcttttacatattttgctgtgcaaaattgttttatatcttgagttactaactaaccacgcgtgttgttcctatgtgcttttctttcattttcaattctggttatatcaagaaaagaataatctacaataataaacggcatttttttttgattctgtactcagtttcttagtgtacagtttaactgggcccaacaacctcgttaaaagtgtaaaatgcatccttttctccagtggaaggattcctggaggaatagggagacagtaattcagggtgaaattataggctgttttttgaagtgaggaggctggccccatatactgattagcaatatttaatatagatgtaaattatgacctcatttttttctccccaaagttttcagttttcaaatgagttgagccataattgcccttggtaggaaaaacaaaacaaaacagtggaactaggcttcctgagcatggccctacacttctgatcaggagcaaagccatccatagacagaggagccggacaaatatggcgcatcagaggtggcttgcgcacatatgcattgaacggtaaagagaaacagcgcttgccttttcactaaagttgactatttttccttcttctcttacacaccgagattttcttgttagcaaggcctgacaagatttaacataaacatgacaaatcatagttgtttgttttgttttgcttttctctttaacactgaagatcatttgtcttaaataggaaaaagaaaatccactccttacttccatatttccaagtacatatctggtttaaactatgttatcaaatcatatttcaccgtgaatattcagtggagaacttctctacctggatgagctagtaatgatttcagatcatgctatccccagaaataaaagcaaaaaataatacctgtgtggaatataggctgtgctttgatttactggtatttaccccaaaataggctgtgtatgggggctgacttaaagatcccttggaaagactcaaaactaccttcactagtaggactcctaagcgctgacctatttttaaatgacacaaattcatgaaactaatgttacaaattcatgcagtttgcactcttagtcatcttcccctagcacaccaatagaatgttagacaaagccagcactgttttgaaaatacagccaaacacgatgacttttgttttgttttctgccgttcttaaaagaaaaaaagataatattgcaactctgactgaaagacttatttttaagaaaacaggttgtgtttggtgctgctaagttctggccagtttatcatctggccttcctgcctattttttacaaaacacgaagacagtgtgtaacctcgacattttgaccttcctttatgtgctagtttagacaggctcctgaatccacacttaattttgcttaacaaaagtcttaatagtaaacctcccctcatgagcttgaagtcaagtgttcttgacttcagatatttctttcctttttttttttttttcctcatcacaactaagagatacacaaactctgaagaagcagaaatggagagaatgcttttaacaaaaaagcatctgatgaaagattttaggcaaacattctcaaaataagagtgatattctggatgtagttattgcagttatctcatgacaaatgaggcctggattggaaggaaaatatagttgtgtagaattaagcattttgataggaatctacaaggtagttgaatataataagcaggtttgggcccccaaactttagaaaatcaaatgcaaaggtgctggcaaaaatgaggtttgagtggctggctgtaagagaaggttaactcctagtaaaaggcatttttagaaataacaattactgaaaactttgaagtatagtgggagtagcaaacaaatacatgttttttttttcttacaaagaactcctaaatcctgagtaagtgccattcattacaataagtctctaaatttaaaaaaaaaaaaatcatatgaggaaatctagctttcccctttacgctgcgtttgatctttgtctaaatagtgttaaaattcctttcattccaattacagaactgagcccactcgcaagttggagccatcagtgggatacgccacattttggaagccccagcatcgtgtacttaccagtgtgttcacaaaatgaaatttgtgtgagagctgtacattaaaaaaaatcatcattattattattatttgcagtcatggagaaccacctacccctgacttctgtttagtctcctttttaaataaaaattactgtgttagagaagaaggctattaaatgtagtagttaactatgcctcttgtctgggggtttcatagagaccggtaggaaagcgcactcctgcttttcgatttatggtgtgtgcaagtaaacaggtgcattgctttcaacctgccatactagttttaaaaattcactgaaattacaaagatacatatatatgcatatatataatggaaagtttcccggaatgcaacaattagcattttaaaatcatatataggcatgcacattctaaatagtactttttcatgcttcattgtttctctggcagataattttactaagaagaaaaatagatattcgactccccttccctaaacaaatccacgggcagaggctccagcggagccgagccccctggttttctcgtaggccctagacggtgttgcatttatcagtgatgtcaaacgtgctcatttgtcagacatagctgtaaatgaaaacaatgtgtggcaaaatacaaagttagttaaatacacaccctctgtgtgattttttgctcccttttcttttttgctcctactcaaaaaaaaaaaaatcacctcctttacatttccctggcttcttgcatgtttcccttttcaaaaaccatgtaataattttttacaatgtatctgacacattaatatattgacatcaaataggcagacattctacttttgcctggcaaataaatctgctacggagacatcatttcctcactgtctcaaagccataactacctgggagtctttcaacacagacccctccgatgggaaatgctgtttattactgaatgcaggatgctcacgctctgatcttttctcccttgtgcctttaccccagtcatttttacttagcaacaccaattctagatacttctgttctgaagtagaaccacccccttgccacactgccagttttcctgctaaaagcagtggacagaagacagatcatggtcaccctcacaaacatggcacacagctgtctcggtagctgcattcccagcatgtcctggtctaaatatctagagttgcctatgacacgttcaaaggttcccaagcacagtacattgggaggcttttgctgctgtggccgttgttttcgtttaggccaacttacttccgtattcacatactcttggctttacgaaatacactcctccagtctactaggccaatcaatatatttaaaagtctgattgccacataagtctctctctctctctttttgttttttgtttgtttgtttttttctgttttggctgccggtagttaaagactgagataggttggaagactaaaatacaggagtacatgagtgacaaccttcagccgtctgatttccatgccggtaaaacacacaaccaagctcttcttagcgctgctaatataaacattcactaagagggaataggaagtgagatttaccagcttcactttgctgatttgcaaggttccccactacgattcactgtcatttgatttttgaaaaataattttgtccgtctctttgaagaaatgtcttagttcttttattttgtttgtttggttttttttagagaagttttatctgcagtgataggctacaatttttatctccgctgattatttgtcaggatgctgaatgaataatttggtcctgtgccttccttgttgttctgaggaaaataagagaaacttggaagtttgtttcactcttagcccatcctaaatctaaaagaagatgtcccaggtccaggcaggccatgtagtagttataaaggaggtggtccaggtccagccacctcaatcaggatttgtttgttttgaagcatttgcttaaaagcggagcaagagtcttaacccaacttgccataacactgcttttctcgcttttgatgtaaatcttcaaaattcagacatcaaacagccccagaaaaggggaattctctccaggcattgctccgccccagctcctgaacaaacccagctctgtctagcatttttttccctagcgggggtaggggacagggtgagagaatttcagtctcccaggctgtctcatgattgttagggcataaagaaacacagtcctgccacaaattgggagcatctttaccctttagagagaaacaaaacaaaactaaacaaacaaatcaaattgctttgcatgaaggcgtagcaaataaaatctcgggctccctgttccctgcaccatttgtaggaggtgagaaatgagggaaacaagagaaaggggaactttaaaagcgggaggcccagaaataatccctgttaccagtctgaatttcacttgctccgtggctaacgtcagacctagtgtgcatgtatgccagaagtaaactaggctcggctgtccatttctttaaaatatgttcacatgtttcctttttgaaaacaattttggggactaaacccaaatggagagatttgaggaaatcgttaatgtcttaacatttgagtatatttataaatgtatcagtctgtgat